European Patent Specification EP 3 402 815 B1, published December 6, 2023. Title: ENDO-S2 MUTANTS AS GLYCOSYNTHASES, METHOD OF MAKING AND USE FOR GLYCOENGINEERING OF GLYCOPRTEINS. Applicant: University of Maryland, College Park Wang, Lai-Xi Yang, Qiang Li, Tiezheng Tong, Xin. The sequence listing filed with the application follows.

SEQUENCE LISTING (24 sequences)

SEQ ID NO: 1 - protein, 843 aa, Streptococcus pyogenes
MDKHLLVKRTLGCVCAATLMGAALATHHDSLNTVKAEEKTVQTGKTDQQVGAKLVQEIREGKRGPLYAGYFRTWHDRASTGIDGKQQHPENTMAEVPKEVDILFVFHDHTASDSPFWSELKDSYVHKLHQQGTALVQTIGVNELNGRTGLSKDYPDTPEGNKALAAAIVKAFVTDRGVDGLDIDIEHEFTNKRTPEEDARALNVFKEIAQLIGKNGSDKSKLLIMDTTLSVENNPIFKGIAEDLDYLLRQYYGSQGGEAEVDTINSDWNQYQNYIDASQFMIGFSFFEESASKGNLWFDVNEYDPNNPEKGKDIEGTRAKKYAEWQPSTGGLKAGIFSYAIDRDGVAHVPSTYKNRTSTNLQRHEVDNISHTDYTVSRKLKTLMTEDKRYDVIDQKDIPDPALREQIIQQVGQYKGDLERYNKTLVLTGDKIQNLKGLEKLSKLQKLELRQLSNVKEITPELLPESMKKDAELVMVGMTGLEKLNLSGLNRQTLDGIDVNSITHLTSFDISHNSLDLSEKSEDRKLLMTLMEQVSNHQKITVKNTAFENQKPKGYYPQTYDTKEGHYDVDNAEHDILTDFVFGTVTKRNTFIGDEEAFAIYKEGAVDGRQYVSKDYTYEAFRKDYKGYKVHLTASNLGETVTSKVTATTDETYLVDVSDGEKVVHHMKLNIGSGAIMMENLAKGAKVIGTSGDFEQAKKIFDGEKSDRFFTWGQTNWIAFDLGEINLAKEWRLFNAETNTEIKTDSSLNVAKGRLQILKDTTIDLEKMDIKNRKEYLSNDENWTDVAQMDDAKAIFNSKLSNVLSRYWRFCVDGGASSYYPQYTELQILGQRLSNDVANTLKD

SEQ ID NO: 2 - protein, 843 aa, Artificial Sequence
  Synthetic Construct
MDKHLLVKRTLGCVCAATLMGAALATHHDSLNTVKAEEKTVQTGKTDQQVGAKLVQEIREGKRGPLYAGYFRTWHDRASTGIDGKQQHPENTMAEVPKEVDILFVFHDHTASDSPFWSELKDSYVHKLHQQGTALVQTIGVNELNGRTGLSKDYPDTPEGNKALAAAIVKAFVTDRGVDGLDIAIEHEFTNKRTPEEDARALNVFKEIAQLIGKNGSDKSKLLIMDTTLSVENNPIFKGIAEDLDYLLRQYYGSQGGEAEVDTINSDWNQYQNYIDASQFMIGFSFFEESASKGNLWFDVNEYDPNNPEKGKDIEGTRAKKYAEWQPSTGGLKAGIFSYAIDRDGVAHVPSTYKNRTSTNLQRHEVDNISHTDYTVSRKLKTLMTEDKRYDVIDQKDIPDPALREQIIQQVGQYKGDLERYNKTLVLTGDKIQNLKGLEKLSKLQKLELRQLSNVKEITPELLPESMKKDAELVMVGMTGLEKLNLSGLNRQTLDGIDVNSITHLTSFDISHNSLDLSEKSEDRKLLMTLMEQVSNHQKITVKNTAFENQKPKGYYPQTYDTKEGHYDVDNAEHDILTDFVFGTVTKRNTFIGDEEAFAIYKEGAVDGRQYVSKDYTYEAFRKDYKGYKVHLTASNLGETVTSKVTATTDETYLVDVSDGEKVVHHMKLNIGSGAIMMENLAKGAKVIGTSGDFEQAKKIFDGEKSDRFFTWGQTNWIAFDLGEINLAKEWRLFNAETNTEIKTDSSLNVAKGRLQILKDTTIDLEKMDIKNRKEYLSNDENWTDVAQMDDAKAIFNSKLSNVLSRYWRFCVDGGASSYYPQYTELQILGQRLSNDVANTLKD

SEQ ID NO: 3 - protein, 843 aa, Artificial Sequence
  Synthetic Construct
MDKHLLVKRTLGCVCAATLMGAALATHHDSLNTVKAEEKTVQTGKTDQQVGAKLVQEIREGKRGPLYAGYFRTWHDRASTGIDGKQQHPENTMAEVPKEVDILFVFHDHTASDSPFWSELKDSYVHKLHQQGTALVQTIGVNELNGRTGLSKDYPDTPEGNKALAAAIVKAFVTDRGVDGLDINIEHEFTNKRTPEEDARALNVFKEIAQLIGKNGSDKSKLLIMDTTLSVENNPIFKGIAEDLDYLLRQYYGSQGGEAEVDTINSDWNQYQNYIDASQFMIGFSFFEESASKGNLWFDVNEYDPNNPEKGKDIEGTRAKKYAEWQPSTGGLKAGIFSYAIDRDGVAHVPSTYKNRTSTNLQRHEVDNISHTDYTVSRKLKTLMTEDKRYDVIDQKDIPDPALREQIIQQVGQYKGDLERYNKTLVLTGDKIQNLKGLEKLSKLQKLELRQLSNVKEITPELLPESMKKDAELVMVGMTGLEKLNLSGLNRQTLDGIDVNSITHLTSFDISHNSLDLSEKSEDRKLLMTLMEQVSNHQKITVKNTAFENQKPKGYYPQTYDTKEGHYDVDNAEHDILTDFVFGTVTKRNTFIGDEEAFAIYKEGAVDGRQYVSKDYTYEAFRKDYKGYKVHLTASNLGETVTSKVTATTDETYLVDVSDGEKVVHHMKLNIGSGAIMMENLAKGAKVIGTSGDFEQAKKIFDGEKSDRFFTWGQTNWIAFDLGEINLAKEWRLFNAETNTEIKTDSSLNVAKGRLQILKDTTIDLEKMDIKNRKEYLSNDENWTDVAQMDDAKAIFNSKLSNVLSRYWRFCVDGGASSYYPQYTELQILGQRLSNDVANTLKD

SEQ ID NO: 4 - protein, 843 aa, Artificial Sequence
  Synthetic Construct
MDKHLLVKRTLGCVCAATLMGAALATHHDSLNTVKAEEKTVQTGKTDQQVGAKLVQEIREGKRGPLYAGYFRTWHDRASTGIDGKQQHPENTMAEVPKEVDILFVFHDHTASDSPFWSELKDSYVHKLHQQGTALVQTIGVNELNGRTGLSKDYPDTPEGNKALAAAIVKAFVTDRGVDGLDIQIEHEFTNKRTPEEDARALNVFKEIAQLIGKNGSDKSKLLIMDTTLSVENNPIFKGIAEDLDYLLRQYYGSQGGEAEVDTINSDWNQYQNYIDASQFMIGFSFFEESASKGNLWFDVNEYDPNNPEKGKDIEGTRAKKYAEWQPSTGGLKAGIFSYAIDRDGVAHVPSTYKNRTSTNLQRHEVDNISHTDYTVSRKLKTLMTEDKRYDVIDQKDIPDPALREQIIQQVGQYKGDLERYNKTLVLTGDKIQNLKGLEKLSKLQKLELRQLSNVKEITPELLPESMKKDAELVMVGMTGLEKLNLSGLNRQTLDGIDVNSITHLTSFDISHNSLDLSEKSEDRKLLMTLMEQVSNHQKITVKNTAFENQKPKGYYPQTYDTKEGHYDVDNAEHDILTDFVFGTVTKRNTFIGDEEAFAIYKEGAVDGRQYVSKDYTYEAFRKDYKGYKVHLTASNLGETVTSKVTATTDETYLVDVSDGEKVVHHMKLNIGSGAIMMENLAKGAKVIGTSGDFEQAKKIFDGEKSDRFFTWGQTNWIAFDLGEINLAKEWRLFNAETNTEIKTDSSLNVAKGRLQILKDTTIDLEKMDIKNRKEYLSNDENWTDVAQMDDAKAIFNSKLSNVLSRYWRFCVDGGASSYYPQYTELQILGQRLSNDVANTLKD

SEQ ID NO: 5 - protein, 843 aa, Artificial Sequence
  Synthetic Construct
MDKHLLVKRTLGCVCAATLMGAALATHHDSLNTVKAEEKTVQTGKTDQQVGAKLVQEIREGKRGPLYAGYFRTWHDRASTGIDGKQQHPENTMAEVPKEVDILFVFHDHTASDSPFWSELKDSYVHKLHQQGTALVQTIGVNELNGRTGLSKDYPDTPEGNKALAAAIVKAFVTDRGVDGLDIRIEHEFTNKRTPEEDARALNVFKEIAQLIGKNGSDKSKLLIMDTTLSVENNPIFKGIAEDLDYLLRQYYGSQGGEAEVDTINSDWNQYQNYIDASQFMIGFSFFEESASKGNLWFDVNEYDPNNPEKGKDIEGTRAKKYAEWQPSTGGLKAGIFSYAIDRDGVAHVPSTYKNRTSTNLQRHEVDNISHTDYTVSRKLKTLMTEDKRYDVIDQKDIPDPALREQIIQQVGQYKGDLERYNKTLVLTGDKIQNLKGLEKLSKLQKLELRQLSNVKEITPELLPESMKKDAELVMVGMTGLEKLNLSGLNRQTLDGIDVNSITHLTSFDISHNSLDLSEKSEDRKLLMTLMEQVSNHQKITVKNTAFENQKPKGYYPQTYDTKEGHYDVDNAEHDILTDFVFGTVTKRNTFIGDEEAFAIYKEGAVDGRQYVSKDYTYEAFRKDYKGYKVHLTASNLGETVTSKVTATTDETYLVDVSDGEKVVHHMKLNIGSGAIMMENLAKGAKVIGTSGDFEQAKKIFDGEKSDRFFTWGQTNWIAFDLGEINLAKEWRLFNAETNTEIKTDSSLNVAKGRLQILKDTTIDLEKMDIKNRKEYLSNDENWTDVAQMDDAKAIFNSKLSNVLSRYWRFCVDGGASSYYPQYTELQILGQRLSNDVANTLKD

SEQ ID NO: 6 - protein, 843 aa, Artificial Sequence
  Synthetic Construct
MDKHLLVKRTLGCVCAATLMGAALATHHDSLNTVKAEEKTVQTGKTDQQVGAKLVQEIREGKRGPLYAGYFRTWHDRASTGIDGKQQHPENTMAEVPKEVDILFVFHDHTASDSPFWSELKDSYVHKLHQQGTALVQTIGVNELNGRTGLSKDYPDTPEGNKALAAAIVKAFVTDRGVDGLDICIEHEFTNKRTPEEDARALNVFKEIAQLIGKNGSDKSKLLIMDTTLSVENNPIFKGIAEDLDYLLRQYYGSQGGEAEVDTINSDWNQYQNYIDASQFMIGFSFFEESASKGNLWFDVNEYDPNNPEKGKDIEGTRAKKYAEWQPSTGGLKAGIFSYAIDRDGVAHVPSTYKNRTSTNLQRHEVDNISHTDYTVSRKLKTLMTEDKRYDVIDQKDIPDPALREQIIQQVGQYKGDLERYNKTLVLTGDKIQNLKGLEKLSKLQKLELRQLSNVKEITPELLPESMKKDAELVMVGMTGLEKLNLSGLNRQTLDGIDVNSITHLTSFDISHNSLDLSEKSEDRKLLMTLMEQVSNHQKITVKNTAFENQKPKGYYPQTYDTKEGHYDVDNAEHDILTDFVFGTVTKRNTFIGDEEAFAIYKEGAVDGRQYVSKDYTYEAFRKDYKGYKVHLTASNLGETVTSKVTATTDETYLVDVSDGEKVVHHMKLNIGSGAIMMENLAKGAKVIGTSGDFEQAKKIFDGEKSDRFFTWGQTNWIAFDLGEINLAKEWRLFNAETNTEIKTDSSLNVAKGRLQILKDTTIDLEKMDIKNRKEYLSNDENWTDVAQMDDAKAIFNSKLSNVLSRYWRFCVDGGASSYYPQYTELQILGQRLSNDVANTLKD

SEQ ID NO: 7 - protein, 843 aa, Artificial Sequence
  Synthetic Construct
MDKHLLVKRTLGCVCAATLMGAALATHHDSLNTVKAEEKTVQTGKTDQQVGAKLVQEIREGKRGPLYAGYFRTWHDRASTGIDGKQQHPENTMAEVPKEVDILFVFHDHTASDSPFWSELKDSYVHKLHQQGTALVQTIGVNELNGRTGLSKDYPDTPEGNKALAAAIVKAFVTDRGVDGLDIMIEHEFTNKRTPEEDARALNVFKEIAQLIGKNGSDKSKLLIMDTTLSVENNPIFKGIAEDLDYLLRQYYGSQGGEAEVDTINSDWNQYQNYIDASQFMIGFSFFEESASKGNLWFDVNEYDPNNPEKGKDIEGTRAKKYAEWQPSTGGLKAGIFSYAIDRDGVAHVPSTYKNRTSTNLQRHEVDNISHTDYTVSRKLKTLMTEDKRYDVIDQKDIPDPALREQIIQQVGQYKGDLERYNKTLVLTGDKIQNLKGLEKLSKLQKLELRQLSNVKEITPELLPESMKKDAELVMVGMTGLEKLNLSGLNRQTLDGIDVNSITHLTSFDISHNSLDLSEKSEDRKLLMTLMEQVSNHQKITVKNTAFENQKPKGYYPQTYDTKEGHYDVDNAEHDILTDFVFGTVTKRNTFIGDEEAFAIYKEGAVDGRQYVSKDYTYEAFRKDYKGYKVHLTASNLGETVTSKVTATTDETYLVDVSDGEKVVHHMKLNIGSGAIMMENLAKGAKVIGTSGDFEQAKKIFDGEKSDRFFTWGQTNWIAFDLGEINLAKEWRLFNAETNTEIKTDSSLNVAKGRLQILKDTTIDLEKMDIKNRKEYLSNDENWTDVAQMDDAKAIFNSKLSNVLSRYWRFCVDGGASSYYPQYTELQILGQRLSNDVANTLKD

SEQ ID NO: 8 - protein, 843 aa, Artificial Sequence
  Synthetic Construct
MDKHLLVKRTLGCVCAATLMGAALATHHDSLNTVKAEEKTVQTGKTDQQVGAKLVQEIREGKRGPLYAGYFRTWHDRASTGIDGKQQHPENTMAEVPKEVDILFVFHDHTASDSPFWSELKDSYVHKLHQQGTALVQTIGVNELNGRTGLSKDYPDTPEGNKALAAAIVKAFVTDRGVDGLDIEIEHEFTNKRTPEEDARALNVFKEIAQLIGKNGSDKSKLLIMDTTLSVENNPIFKGIAEDLDYLLRQYYGSQGGEAEVDTINSDWNQYQNYIDASQFMIGFSFFEESASKGNLWFDVNEYDPNNPEKGKDIEGTRAKKYAEWQPSTGGLKAGIFSYAIDRDGVAHVPSTYKNRTSTNLQRHEVDNISHTDYTVSRKLKTLMTEDKRYDVIDQKDIPDPALREQIIQQVGQYKGDLERYNKTLVLTGDKIQNLKGLEKLSKLQKLELRQLSNVKEITPELLPESMKKDAELVMVGMTGLEKLNLSGLNRQTLDGIDVNSITHLTSFDISHNSLDLSEKSEDRKLLMTLMEQVSNHQKITVKNTAFENQKPKGYYPQTYDTKEGHYDVDNAEHDILTDFVFGTVTKRNTFIGDEEAFAIYKEGAVDGRQYVSKDYTYEAFRKDYKGYKVHLTASNLGETVTSKVTATTDETYLVDVSDGEKVVHHMKLNIGSGAIMMENLAKGAKVIGTSGDFEQAKKIFDGEKSDRFFTWGQTNWIAFDLGEINLAKEWRLFNAETNTEIKTDSSLNVAKGRLQILKDTTIDLEKMDIKNRKEYLSNDENWTDVAQMDDAKAIFNSKLSNVLSRYWRFCVDGGASSYYPQYTELQILGQRLSNDVANTLKD

SEQ ID NO: 9 - protein, 843 aa, Artificial Sequence
  Synthetic Construct
MDKHLLVKRTLGCVCAATLMGAALATHHDSLNTVKAEEKTVQTGKTDQQVGAKLVQEIREGKRGPLYAGYFRTWHDRASTGIDGKQQHPENTMAEVPKEVDILFVFHDHTASDSPFWSELKDSYVHKLHQQGTALVQTIGVNELNGRTGLSKDYPDTPEGNKALAAAIVKAFVTDRGVDGLDIGIEHEFTNKRTPEEDARALNVFKEIAQLIGKNGSDKSKLLIMDTTLSVENNPIFKGIAEDLDYLLRQYYGSQGGEAEVDTINSDWNQYQNYIDASQFMIGFSFFEESASKGNLWFDVNEYDPNNPEKGKDIEGTRAKKYAEWQPSTGGLKAGIFSYAIDRDGVAHVPSTYKNRTSTNLQRHEVDNISHTDYTVSRKLKTLMTEDKRYDVIDQKDIPDPALREQIIQQVGQYKGDLERYNKTLVLTGDKIQNLKGLEKLSKLQKLELRQLSNVKEITPELLPESMKKDAELVMVGMTGLEKLNLSGLNRQTLDGIDVNSITHLTSFDISHNSLDLSEKSEDRKLLMTLMEQVSNHQKITVKNTAFENQKPKGYYPQTYDTKEGHYDVDNAEHDILTDFVFGTVTKRNTFIGDEEAFAIYKEGAVDGRQYVSKDYTYEAFRKDYKGYKVHLTASNLGETVTSKVTATTDETYLVDVSDGEKVVHHMKLNIGSGAIMMENLAKGAKVIGTSGDFEQAKKIFDGEKSDRFFTWGQTNWIAFDLGEINLAKEWRLFNAETNTEIKTDSSLNVAKGRLQILKDTTIDLEKMDIKNRKEYLSNDENWTDVAQMDDAKAIFNSKLSNVLSRYWRFCVDGGASSYYPQYTELQILGQRLSNDVANTLKD

SEQ ID NO: 10 - protein, 843 aa, Artificial Sequence
  Synthetic Construct
MDKHLLVKRTLGCVCAATLMGAALATHHDSLNTVKAEEKTVQTGKTDQQVGAKLVQEIREGKRGPLYAGYFRTWHDRASTGIDGKQQHPENTMAEVPKEVDILFVFHDHTASDSPFWSELKDSYVHKLHQQGTALVQTIGVNELNGRTGLSKDYPDTPEGNKALAAAIVKAFVTDRGVDGLDIHIEHEFTNKRTPEEDARALNVFKEIAQLIGKNGSDKSKLLIMDTTLSVENNPIFKGIAEDLDYLLRQYYGSQGGEAEVDTINSDWNQYQNYIDASQFMIGFSFFEESASKGNLWFDVNEYDPNNPEKGKDIEGTRAKKYAEWQPSTGGLKAGIFSYAIDRDGVAHVPSTYKNRTSTNLQRHEVDNISHTDYTVSRKLKTLMTEDKRYDVIDQKDIPDPALREQIIQQVGQYKGDLERYNKTLVLTGDKIQNLKGLEKLSKLQKLELRQLSNVKEITPELLPESMKKDAELVMVGMTGLEKLNLSGLNRQTLDGIDVNSITHLTSFDISHNSLDLSEKSEDRKLLMTLMEQVSNHQKITVKNTAFENQKPKGYYPQTYDTKEGHYDVDNAEHDILTDFVFGTVTKRNTFIGDEEAFAIYKEGAVDGRQYVSKDYTYEAFRKDYKGYKVHLTASNLGETVTSKVTATTDETYLVDVSDGEKVVHHMKLNIGSGAIMMENLAKGAKVIGTSGDFEQAKKIFDGEKSDRFFTWGQTNWIAFDLGEINLAKEWRLFNAETNTEIKTDSSLNVAKGRLQILKDTTIDLEKMDIKNRKEYLSNDENWTDVAQMDDAKAIFNSKLSNVLSRYWRFCVDGGASSYYPQYTELQILGQRLSNDVANTLKD

SEQ ID NO: 11 - protein, 843 aa, Artificial Sequence
  Synthetic Construct
MDKHLLVKRTLGCVCAATLMGAALATHHDSLNTVKAEEKTVQTGKTDQQVGAKLVQEIREGKRGPLYAGYFRTWHDRASTGIDGKQQHPENTMAEVPKEVDILFVFHDHTASDSPFWSELKDSYVHKLHQQGTALVQTIGVNELNGRTGLSKDYPDTPEGNKALAAAIVKAFVTDRGVDGLDIIIEHEFTNKRTPEEDARALNVFKEIAQLIGKNGSDKSKLLIMDTTLSVENNPIFKGIAEDLDYLLRQYYGSQGGEAEVDTINSDWNQYQNYIDASQFMIGFSFFEESASKGNLWFDVNEYDPNNPEKGKDIEGTRAKKYAEWQPSTGGLKAGIFSYAIDRDGVAHVPSTYKNRTSTNLQRHEVDNISHTDYTVSRKLKTLMTEDKRYDVIDQKDIPDPALREQIIQQVGQYKGDLERYNKTLVLTGDKIQNLKGLEKLSKLQKLELRQLSNVKEITPELLPESMKKDAELVMVGMTGLEKLNLSGLNRQTLDGIDVNSITHLTSFDISHNSLDLSEKSEDRKLLMTLMEQVSNHQKITVKNTAFENQKPKGYYPQTYDTKEGHYDVDNAEHDILTDFVFGTVTKRNTFIGDEEAFAIYKEGAVDGRQYVSKDYTYEAFRKDYKGYKVHLTASNLGETVTSKVTATTDETYLVDVSDGEKVVHHMKLNIGSGAIMMENLAKGAKVIGTSGDFEQAKKIFDGEKSDRFFTWGQTNWIAFDLGEINLAKEWRLFNAETNTEIKTDSSLNVAKGRLQILKDTTIDLEKMDIKNRKEYLSNDENWTDVAQMDDAKAIFNSKLSNVLSRYWRFCVDGGASSYYPQYTELQILGQRLSNDVANTLKD

SEQ ID NO: 12 - protein, 843 aa, Artificial Sequence
  Synthetic Construct
MDKHLLVKRTLGCVCAATLMGAALATHHDSLNTVKAEEKTVQTGKTDQQVGAKLVQEIREGKRGPLYAGYFRTWHDRASTGIDGKQQHPENTMAEVPKEVDILFVFHDHTASDSPFWSELKDSYVHKLHQQGTALVQTIGVNELNGRTGLSKDYPDTPEGNKALAAAIVKAFVTDRGVDGLDILIEHEFTNKRTPEEDARALNVFKEIAQLIGKNGSDKSKLLIMDTTLSVENNPIFKGIAEDLDYLLRQYYGSQGGEAEVDTINSDWNQYQNYIDASQFMIGFSFFEESASKGNLWFDVNEYDPNNPEKGKDIEGTRAKKYAEWQPSTGGLKAGIFSYAIDRDGVAHVPSTYKNRTSTNLQRHEVDNISHTDYTVSRKLKTLMTEDKRYDVIDQKDIPDPALREQIIQQVGQYKGDLERYNKTLVLTGDKIQNLKGLEKLSKLQKLELRQLSNVKEITPELLPESMKKDAELVMVGMTGLEKLNLSGLNRQTLDGIDVNSITHLTSFDISHNSLDLSEKSEDRKLLMTLMEQVSNHQKITVKNTAFENQKPKGYYPQTYDTKEGHYDVDNAEHDILTDFVFGTVTKRNTFIGDEEAFAIYKEGAVDGRQYVSKDYTYEAFRKDYKGYKVHLTASNLGETVTSKVTATTDETYLVDVSDGEKVVHHMKLNIGSGAIMMENLAKGAKVIGTSGDFEQAKKIFDGEKSDRFFTWGQTNWIAFDLGEINLAKEWRLFNAETNTEIKTDSSLNVAKGRLQILKDTTIDLEKMDIKNRKEYLSNDENWTDVAQMDDAKAIFNSKLSNVLSRYWRFCVDGGASSYYPQYTELQILGQRLSNDVANTLKD

SEQ ID NO: 13 - protein, 843 aa, Artificial Sequence
  Synthetic Construct
MDKHLLVKRTLGCVCAATLMGAALATHHDSLNTVKAEEKTVQTGKTDQQVGAKLVQEIREGKRGPLYAGYFRTWHDRASTGIDGKQQHPENTMAEVPKEVDILFVFHDHTASDSPFWSELKDSYVHKLHQQGTALVQTIGVNELNGRTGLSKDYPDTPEGNKALAAAIVKAFVTDRGVDGLDIKIEHEFTNKRTPEEDARALNVFKEIAQLIGKNGSDKSKLLIMDTTLSVENNPIFKGIAEDLDYLLRQYYGSQGGEAEVDTINSDWNQYQNYIDASQFMIGFSFFEESASKGNLWFDVNEYDPNNPEKGKDIEGTRAKKYAEWQPSTGGLKAGIFSYAIDRDGVAHVPSTYKNRTSTNLQRHEVDNISHTDYTVSRKLKTLMTEDKRYDVIDQKDIPDPALREQIIQQVGQYKGDLERYNKTLVLTGDKIQNLKGLEKLSKLQKLELRQLSNVKEITPELLPESMKKDAELVMVGMTGLEKLNLSGLNRQTLDGIDVNSITHLTSFDISHNSLDLSEKSEDRKLLMTLMEQVSNHQKITVKNTAFENQKPKGYYPQTYDTKEGHYDVDNAEHDILTDFVFGTVTKRNTFIGDEEAFAIYKEGAVDGRQYVSKDYTYEAFRKDYKGYKVHLTASNLGETVTSKVTATTDETYLVDVSDGEKVVHHMKLNIGSGAIMMENLAKGAKVIGTSGDFEQAKKIFDGEKSDRFFTWGQTNWIAFDLGEINLAKEWRLFNAETNTEIKTDSSLNVAKGRLQILKDTTIDLEKMDIKNRKEYLSNDENWTDVAQMDDAKAIFNSKLSNVLSRYWRFCVDGGASSYYPQYTELQILGQRLSNDVANTLKD

SEQ ID NO: 14 - protein, 843 aa, Artificial Sequence
  Synthetic Construct
MDKHLLVKRTLGCVCAATLMGAALATHHDSLNTVKAEEKTVQTGKTDQQVGAKLVQEIREGKRGPLYAGYFRTWHDRASTGIDGKQQHPENTMAEVPKEVDILFVFHDHTASDSPFWSELKDSYVHKLHQQGTALVQTIGVNELNGRTGLSKDYPDTPEGNKALAAAIVKAFVTDRGVDGLDIFIEHEFTNKRTPEEDARALNVFKEIAQLIGKNGSDKSKLLIMDTTLSVENNPIFKGIAEDLDYLLRQYYGSQGGEAEVDTINSDWNQYQNYIDASQFMIGFSFFEESASKGNLWFDVNEYDPNNPEKGKDIEGTRAKKYAEWQPSTGGLKAGIFSYAIDRDGVAHVPSTYKNRTSTNLQRHEVDNISHTDYTVSRKLKTLMTEDKRYDVIDQKDIPDPALREQIIQQVGQYKGDLERYNKTLVLTGDKIQNLKGLEKLSKLQKLELRQLSNVKEITPELLPESMKKDAELVMVGMTGLEKLNLSGLNRQTLDGIDVNSITHLTSFDISHNSLDLSEKSEDRKLLMTLMEQVSNHQKITVKNTAFENQKPKGYYPQTYDTKEGHYDVDNAEHDILTDFVFGTVTKRNTFIGDEEAFAIYKEGAVDGRQYVSKDYTYEAFRKDYKGYKVHLTASNLGETVTSKVTATTDETYLVDVSDGEKVVHHMKLNIGSGAIMMENLAKGAKVIGTSGDFEQAKKIFDGEKSDRFFTWGQTNWIAFDLGEINLAKEWRLFNAETNTEIKTDSSLNVAKGRLQILKDTTIDLEKMDIKNRKEYLSNDENWTDVAQMDDAKAIFNSKLSNVLSRYWRFCVDGGASSYYPQYTELQILGQRLSNDVANTLKD

SEQ ID NO: 15 - protein, 843 aa, Artificial Sequence
  Synthetic Construct
MDKHLLVKRTLGCVCAATLMGAALATHHDSLNTVKAEEKTVQTGKTDQQVGAKLVQEIREGKRGPLYAGYFRTWHDRASTGIDGKQQHPENTMAEVPKEVDILFVFHDHTASDSPFWSELKDSYVHKLHQQGTALVQTIGVNELNGRTGLSKDYPDTPEGNKALAAAIVKAFVTDRGVDGLDIPIEHEFTNKRTPEEDARALNVFKEIAQLIGKNGSDKSKLLIMDTTLSVENNPIFKGIAEDLDYLLRQYYGSQGGEAEVDTINSDWNQYQNYIDASQFMIGFSFFEESASKGNLWFDVNEYDPNNPEKGKDIEGTRAKKYAEWQPSTGGLKAGIFSYAIDRDGVAHVPSTYKNRTSTNLQRHEVDNISHTDYTVSRKLKTLMTEDKRYDVIDQKDIPDPALREQIIQQVGQYKGDLERYNKTLVLTGDKIQNLKGLEKLSKLQKLELRQLSNVKEITPELLPESMKKDAELVMVGMTGLEKLNLSGLNRQTLDGIDVNSITHLTSFDISHNSLDLSEKSEDRKLLMTLMEQVSNHQKITVKNTAFENQKPKGYYPQTYDTKEGHYDVDNAEHDILTDFVFGTVTKRNTFIGDEEAFAIYKEGAVDGRQYVSKDYTYEAFRKDYKGYKVHLTASNLGETVTSKVTATTDETYLVDVSDGEKVVHHMKLNIGSGAIMMENLAKGAKVIGTSGDFEQAKKIFDGEKSDRFFTWGQTNWIAFDLGEINLAKEWRLFNAETNTEIKTDSSLNVAKGRLQILKDTTIDLEKMDIKNRKEYLSNDENWTDVAQMDDAKAIFNSKLSNVLSRYWRFCVDGGASSYYPQYTELQILGQRLSNDVANTLKD

SEQ ID NO: 16 - protein, 843 aa, Artificial Sequence
  Synthetic Construct
MDKHLLVKRTLGCVCAATLMGAALATHHDSLNTVKAEEKTVQTGKTDQQVGAKLVQEIREGKRGPLYAGYFRTWHDRASTGIDGKQQHPENTMAEVPKEVDILFVFHDHTASDSPFWSELKDSYVHKLHQQGTALVQTIGVNELNGRTGLSKDYPDTPEGNKALAAAIVKAFVTDRGVDGLDISIEHEFTNKRTPEEDARALNVFKEIAQLIGKNGSDKSKLLIMDTTLSVENNPIFKGIAEDLDYLLRQYYGSQGGEAEVDTINSDWNQYQNYIDASQFMIGFSFFEESASKGNLWFDVNEYDPNNPEKGKDIEGTRAKKYAEWQPSTGGLKAGIFSYAIDRDGVAHVPSTYKNRTSTNLQRHEVDNISHTDYTVSRKLKTLMTEDKRYDVIDQKDIPDPALREQIIQQVGQYKGDLERYNKTLVLTGDKIQNLKGLEKLSKLQKLELRQLSNVKEITPELLPESMKKDAELVMVGMTGLEKLNLSGLNRQTLDGIDVNSITHLTSFDISHNSLDLSEKSEDRKLLMTLMEQVSNHQKITVKNTAFENQKPKGYYPQTYDTKEGHYDVDNAEHDILTDFVFGTVTKRNTFIGDEEAFAIYKEGAVDGRQYVSKDYTYEAFRKDYKGYKVHLTASNLGETVTSKVTATTDETYLVDVSDGEKVVHHMKLNIGSGAIMMENLAKGAKVIGTSGDFEQAKKIFDGEKSDRFFTWGQTNWIAFDLGEINLAKEWRLFNAETNTEIKTDSSLNVAKGRLQILKDTTIDLEKMDIKNRKEYLSNDENWTDVAQMDDAKAIFNSKLSNVLSRYWRFCVDGGASSYYPQYTELQILGQRLSNDVANTLKD

SEQ ID NO: 17 - protein, 843 aa, Artificial Sequence
  Synthetic Construct
MDKHLLVKRTLGCVCAATLMGAALATHHDSLNTVKAEEKTVQTGKTDQQVGAKLVQEIREGKRGPLYAGYFRTWHDRASTGIDGKQQHPENTMAEVPKEVDILFVFHDHTASDSPFWSELKDSYVHKLHQQGTALVQTIGVNELNGRTGLSKDYPDTPEGNKALAAAIVKAFVTDRGVDGLDITIEHEFTNKRTPEEDARALNVFKEIAQLIGKNGSDKSKLLIMDTTLSVENNPIFKGIAEDLDYLLRQYYGSQGGEAEVDTINSDWNQYQNYIDASQFMIGFSFFEESASKGNLWFDVNEYDPNNPEKGKDIEGTRAKKYAEWQPSTGGLKAGIFSYAIDRDGVAHVPSTYKNRTSTNLQRHEVDNISHTDYTVSRKLKTLMTEDKRYDVIDQKDIPDPALREQIIQQVGQYKGDLERYNKTLVLTGDKIQNLKGLEKLSKLQKLELRQLSNVKEITPELLPESMKKDAELVMVGMTGLEKLNLSGLNRQTLDGIDVNSITHLTSFDISHNSLDLSEKSEDRKLLMTLMEQVSNHQKITVKNTAFENQKPKGYYPQTYDTKEGHYDVDNAEHDILTDFVFGTVTKRNTFIGDEEAFAIYKEGAVDGRQYVSKDYTYEAFRKDYKGYKVHLTASNLGETVTSKVTATTDETYLVDVSDGEKVVHHMKLNIGSGAIMMENLAKGAKVIGTSGDFEQAKKIFDGEKSDRFFTWGQTNWIAFDLGEINLAKEWRLFNAETNTEIKTDSSLNVAKGRLQILKDTTIDLEKMDIKNRKEYLSNDENWTDVAQMDDAKAIFNSKLSNVLSRYWRFCVDGGASSYYPQYTELQILGQRLSNDVANTLKD

SEQ ID NO: 18 - protein, 843 aa, Artificial Sequence
  Synthetic Construct
MDKHLLVKRTLGCVCAATLMGAALATHHDSLNTVKAEEKTVQTGKTDQQVGAKLVQEIREGKRGPLYAGYFRTWHDRASTGIDGKQQHPENTMAEVPKEVDILFVFHDHTASDSPFWSELKDSYVHKLHQQGTALVQTIGVNELNGRTGLSKDYPDTPEGNKALAAAIVKAFVTDRGVDGLDIWIEHEFTNKRTPEEDARALNVFKEIAQLIGKNGSDKSKLLIMDTTLSVENNPIFKGIAEDLDYLLRQYYGSQGGEAEVDTINSDWNQYQNYIDASQFMIGFSFFEESASKGNLWFDVNEYDPNNPEKGKDIEGTRAKKYAEWQPSTGGLKAGIFSYAIDRDGVAHVPSTYKNRTSTNLQRHEVDNISHTDYTVSRKLKTLMTEDKRYDVIDQKDIPDPALREQIIQQVGQYKGDLERYNKTLVLTGDKIQNLKGLEKLSKLQKLELRQLSNVKEITPELLPESMKKDAELVMVGMTGLEKLNLSGLNRQTLDGIDVNSITHLTSFDISHNSLDLSEKSEDRKLLMTLMEQVSNHQKITVKNTAFENQKPKGYYPQTYDTKEGHYDVDNAEHDILTDFVFGTVTKRNTFIGDEEAFAIYKEGAVDGRQYVSKDYTYEAFRKDYKGYKVHLTASNLGETVTSKVTATTDETYLVDVSDGEKVVHHMKLNIGSGAIMMENLAKGAKVIGTSGDFEQAKKIFDGEKSDRFFTWGQTNWIAFDLGEINLAKEWRLFNAETNTEIKTDSSLNVAKGRLQILKDTTIDLEKMDIKNRKEYLSNDENWTDVAQMDDAKAIFNSKLSNVLSRYWRFCVDGGASSYYPQYTELQILGQRLSNDVANTLKD

SEQ ID NO: 19 - protein, 843 aa, Artificial Sequence
  Synthetic Construct
MDKHLLVKRTLGCVCAATLMGAALATHHDSLNTVKAEEKTVQTGKTDQQVGAKLVQEIREGKRGPLYAGYFRTWHDRASTGIDGKQQHPENTMAEVPKEVDILFVFHDHTASDSPFWSELKDSYVHKLHQQGTALVQTIGVNELNGRTGLSKDYPDTPEGNKALAAAIVKAFVTDRGVDGLDIYIEHEFTNKRTPEEDARALNVFKEIAQLIGKNGSDKSKLLIMDTTLSVENNPIFKGIAEDLDYLLRQYYGSQGGEAEVDTINSDWNQYQNYIDASQFMIGFSFFEESASKGNLWFDVNEYDPNNPEKGKDIEGTRAKKYAEWQPSTGGLKAGIFSYAIDRDGVAHVPSTYKNRTSTNLQRHEVDNISHTDYTVSRKLKTLMTEDKRYDVIDQKDIPDPALREQIIQQVGQYKGDLERYNKTLVLTGDKIQNLKGLEKLSKLQKLELRQLSNVKEITPELLPESMKKDAELVMVGMTGLEKLNLSGLNRQTLDGIDVNSITHLTSFDISHNSLDLSEKSEDRKLLMTLMEQVSNHQKITVKNTAFENQKPKGYYPQTYDTKEGHYDVDNAEHDILTDFVFGTVTKRNTFIGDEEAFAIYKEGAVDGRQYVSKDYTYEAFRKDYKGYKVHLTASNLGETVTSKVTATTDETYLVDVSDGEKVVHHMKLNIGSGAIMMENLAKGAKVIGTSGDFEQAKKIFDGEKSDRFFTWGQTNWIAFDLGEINLAKEWRLFNAETNTEIKTDSSLNVAKGRLQILKDTTIDLEKMDIKNRKEYLSNDENWTDVAQMDDAKAIFNSKLSNVLSRYWRFCVDGGASSYYPQYTELQILGQRLSNDVANTLKD

SEQ ID NO: 20 - protein, 843 aa, Artificial Sequence
  Synthetic Construct
MDKHLLVKRTLGCVCAATLMGAALATHHDSLNTVKAEEKTVQTGKTDQQVGAKLVQEIREGKRGPLYAGYFRTWHDRASTGIDGKQQHPENTMAEVPKEVDILFVFHDHTASDSPFWSELKDSYVHKLHQQGTALVQTIGVNELNGRTGLSKDYPDTPEGNKALAAAIVKAFVTDRGVDGLDIVIEHEFTNKRTPEEDARALNVFKEIAQLIGKNGSDKSKLLIMDTTLSVENNPIFKGIAEDLDYLLRQYYGSQGGEAEVDTINSDWNQYQNYIDASQFMIGFSFFEESASKGNLWFDVNEYDPNNPEKGKDIEGTRAKKYAEWQPSTGGLKAGIFSYAIDRDGVAHVPSTYKNRTSTNLQRHEVDNISHTDYTVSRKLKTLMTEDKRYDVIDQKDIPDPALREQIIQQVGQYKGDLERYNKTLVLTGDKIQNLKGLEKLSKLQKLELRQLSNVKEITPELLPESMKKDAELVMVGMTGLEKLNLSGLNRQTLDGIDVNSITHLTSFDISHNSLDLSEKSEDRKLLMTLMEQVSNHQKITVKNTAFENQKPKGYYPQTYDTKEGHYDVDNAEHDILTDFVFGTVTKRNTFIGDEEAFAIYKEGAVDGRQYVSKDYTYEAFRKDYKGYKVHLTASNLGETVTSKVTATTDETYLVDVSDGEKVVHHMKLNIGSGAIMMENLAKGAKVIGTSGDFEQAKKIFDGEKSDRFFTWGQTNWIAFDLGEINLAKEWRLFNAETNTEIKTDSSLNVAKGRLQILKDTTIDLEKMDIKNRKEYLSNDENWTDVAQMDDAKAIFNSKLSNVLSRYWRFCVDGGASSYYPQYTELQILGQRLSNDVANTLKD

SEQ ID NO: 21 - protein, 995 aa, Streptococcus pyogenes
MDKHLLVKRTLGCVCAATLMGAALATHHDSLNTVKAEEKTVQVQKGLPSIDSLHYLSENSKKEFKEELSKAGQESQKVKEILAKAQQADKQAQELAKMKIPEKIPMKPLHGPLYGGYFRTWHDKTSDPTEKDKVNSMGELPKEVDLAFIFHDWTKDYSLFWKELATKHVPKLNKQGTRVIRTIPWRFLAGGDNSGIAEDTSKYPNTPEGNKALAKAIVDEYVYKYNLDGLDVDVEHDSIPKVDKKEDTAGVERSIQVFEEIGKLIGPKGVDKSRLFIMDSTYMADKNPLIERGAPYINLLLVQVYGSQGEKGGWEPVSNRPEKTMEERWQGYSKYIRPEQYMIGFSFYEENAQEGNLWYDINSRKDEDKANGINTDITGTRAERYARWQPKTGGVKGGIFSYAIDRDGVAHQPKKYAKQKEFKDATDNIFHSDYSVSKALKTVMLKDKSYDLIDEKDFPDKALREAVMAQVGTRKGDLERFNGTLRLDNPAIQSLEGLNKFKKLAQLDLIGLSRITKLDRSVLPANMKPGKDTLETVLETYKKDNKEEPATIPPVSLKVSGLTGLKELDLSGFDRETLAGLDAATLTSLEKVDISGNKLDLAPGTENRQIFDTMLSTISNHVGSNEQTVKFDKQKPTGHYPDTYGKTSLRLPVANEKVDLQSQLLFGTVTNQGTLINSEADYKAYQNHKIAGRSFVDSNYHYNNFKVSYENYTVKVTDSTLGTTTDKTLATDKEETYKVDFFSPADKTKAVHTAKVIVGDEKTMMVNLAEGATVIGGSADPVNARKVFDGQLGSETDNISLGWDSKQSIIFKLKEDGLIKHWRFFNDSARNPETTNKPIQEASLQIFNIKDYNLDNLLENPNKFDDEKYWITVDTYSAQGERATAFSNTLNNITSKYWRVVFDTKGDRYSSPVVPELQILGYPLPNADTIMKTVTTAKELSQQKDKFSQKMLDELKIKEMALETSLNSKIFDVTAINANAGVLKDCIEKRQLLKK

SEQ ID NO: 22 - protein, 231 aa, Artificial Sequence
  Synthetic Construct
LGSGKILHNQNVNSWGPITVTPTTDGGETRFDGQIIVQMENDPVVAKAAANLAGKHAESSVVVQLDSDGNYRVVYGDPSKLDGKLRWQLVGHGRDHSETNNTRLSGYSADELAVKLAKFQQSFNQAENINNKPDHISIVGCSLVSDDKQKGFGHQFINAMDANGLRVDVSVRSSELAVDEAGRKHTKDANGDWVQKAENNKVSLSWDAQLEGGSGGSGNSGHHHHHHHHHH

SEQ ID NO: 23 - DNA, 52 bp, Artificial Sequence
  Synthetic Construct
  misc_feature (19)..(21): n is a, c, g, or t
cgtaaattcgtgctcaatnnnaatatctagtccatcgacaccacgatcagtt

SEQ ID NO: 24 - DNA, 52 bp, Artificial Sequence
  synthetic construct
  misc_feature (32)..(34): n is a, c, g, or t
aactgatcgtggtgtcgatggactagatattnnnattgagcacgaatttacg